European Patent Application EP 4 202 045 A1, published June 28, 2023. Title: SYNTHETIC TRANSFER RNA WITH MODIFIED NUCLEOTIDES. Applicant: UNIVERSITAET HAMBURG. The sequence listing filed with the application follows.

SEQUENCE LISTING (38 sequences)

SEQ ID NO: 1 - RNA, 17 nt, Artificial Sequence
  Anticodon arm
  misc_feature 6..12: /note="n = A, C, G or U, or any modified base"
  misc_feature 8..10: /note="anticodon"
gcaggnnnnnnnccugu

SEQ ID NO: 2 - RNA, 18 nt, Artificial Sequence
  Anticodon arm
  misc_feature 6..13: /note="n = A, C, G or U, or any modified base"
  misc_feature 8..11: /note="extended (4nt) anticodon"
gcaggnnnnnnnnccugu

SEQ ID NO: 3 - RNA, 19 nt, Artificial Sequence
  Anticodon arm
  misc_feature 6..14: /note="n = A, C, G or U, or any modified base"
  misc_feature 8..12: /note="extended (5nt) anticodon"
gcaggnnnnnnnnnccugu

SEQ ID NO: 4 - RNA, 20 nt, Artificial Sequence
  Anticodon arm
  misc_feature 6..15: /note="n = A, C, G or U, or any modified base"
  misc_feature 8..13: /note="extended (6nt) anticodon"
gcaggnnnnnnnnnnccugu

SEQ ID NO: 5 - RNA, 17 nt, Artificial Sequence
  Anticodon arm
  misc_feature 6..12: /note="n = A, C, G or U, or any modified base"
  misc_feature 8..10: /note="anticodon"
uugggnnnnnnncucaa

SEQ ID NO: 6 - RNA, 18 nt, Artificial Sequence
  Anticodon arm
  misc_feature 6..13: /note="n = A, C, G or U, or any modified base"
  misc_feature 8..11: /note="extended (4nt) anticodon"
uugggnnnnnnnncucaa

SEQ ID NO: 7 - RNA, 19 nt, Artificial Sequence
  Anticodon arm
  misc_difference 6..14: /note="n = A, C, G or U, or any modified base"
  misc_feature 8..12: /note="extended (5nt) anticodon"
uugggnnnnnnnnncucaa

SEQ ID NO: 8 - RNA, 20 nt, Artificial Sequence
  Anticodon arm
  misc_feature 6..15: /note="n = A, C, G or U, or any modified base"
  misc_feature 8..13: /note="extended (6nt) anticodon"
uugggnnnnnnnnnncucaa

SEQ ID NO: 9 - RNA, 17 nt, Artificial Sequence
  Anticodon arm
  misc_feature 6..12: /note="n = A, C, G or U, or any modified base"
  misc_feature 8..10: /note="anticodon"
uuggannnnnnnuucaa

SEQ ID NO: 10 - RNA, 18 nt, Artificial Sequence
  Anticodon arm
  misc_feature 6..13: /note="n = A, C, G or U, or any modified base"
  misc_feature 8..11: /note="extended (4nt) anticodon"
uuggannnnnnnnuucaa

SEQ ID NO: 11 - RNA, 19 nt, Artificial Sequence
  Anticodon arm
  misc_feature 6..14: /note="n = A, C, G or U, or any modified base"
  misc_feature 8..12: /note="extended (5nt) anticodon"
uuggannnnnnnnnuucaa

SEQ ID NO: 12 - RNA, 20 nt, Artificial Sequence
  Anticodon arm
  misc_feature 6..15: /note="n = A, C, G or U, or any modified base"
  misc_feature 8..13: /note="extended (6nt) anticodon"
uuggannnnnnnnnnuucaa

SEQ ID NO: 13 - RNA, 17 nt, Artificial Sequence
  Anticodon arm
  misc_feature 6..12: /note="n = A, C, G or U, or any modified base"
  misc_feature 8..10: /note="anticodon"
auggunnnnnnnaccau

SEQ ID NO: 14 - RNA, 18 nt, Artificial Sequence
  Anticodon arm
  misc_feature 6..13: /note="n = A, C, G or U, or any modified base"
  misc_feature 8..11: /note="extended (4nt) anticodon"
auggunnnnnnnnaccau

SEQ ID NO: 15 - RNA, 19 nt, Artificial Sequence
  Anticodon arm
  misc_feature 6..14: /note="n = A, C, G or U, or any modified base"
  misc_feature 8..12: /note="extended (5nt) anticodon"
auggunnnnnnnnnaccau

SEQ ID NO: 16 - RNA, 20 nt, Artificial Sequence
  Anticodon arm
  misc_feature 6..15: /note="n = A, C, G or U, or any modified base"
  misc_feature 8..13: /note="extended (6nt) anticodon"
auggunnnnnnnnnnaccau

SEQ ID NO: 17 - RNA, 17 nt, Artificial Sequence
  Anticodon arm
  misc_feature 8..10: /note="n = A, C, G or U, or any modified base" /note="anticodon"
gcaggcunnnaaccugu

SEQ ID NO: 18 - RNA, 18 nt, Artificial Sequence
  Anticodon arm
  misc_feature 8..11: /note="n = A, C, G or U, or any modified base" /note="extended (4nt) anticodon"
gcaggcunnnnaaccugu

SEQ ID NO: 19 - RNA, 19 nt, Artificial Sequence
  Anticodon arm
  misc_feature 8..12: /note="n = A, C, G or U, or any modified base" /note="extended (5nt) anticodon"
gcaggcunnnnnaaccugu

SEQ ID NO: 20 - RNA, 20 nt, Artificial Sequence
  Anticodon arm
  misc_feature 8..13: /note="n = A, C, G or U, or any modified base" /note="extended (6nt) anticodon"
gcaggcunnnnnnaaccugu

SEQ ID NO: 21 - RNA, 17 nt, Artificial Sequence
  Anticodon arm
  misc_feature 8..10: /note="n = A, C, G or U, or any modified base" /note="anticodon"
uugggcunnnaacucaa

SEQ ID NO: 22 - RNA, 18 nt, Artificial Sequence
  anticodon arm
  misc_feature 8..11: /note="n = A, C, G or U, or any modified base" /note="extended (4nt) anticodon"
uugggcunnnnaacucaa

SEQ ID NO: 23 - RNA, 19 nt, Artificial Sequence
  Anticodon arm
  misc_feature 8..12: /note="n = A, C, G or U, or any modified base" /note="extended (5nt) anticodon"
uugggcunnnnnaacucaa

SEQ ID NO: 24 - RNA, 20 nt, Artificial Sequence
  Anticodon arm
  misc_feature 8..13: /note="n = A, C, G or U, or any modified base" /note="extended (6nt) anticodon"
uugggcunnnnnnaacucaa

SEQ ID NO: 25 - RNA, 17 nt, Artificial Sequence
  Anticodon arm
  misc_feature 8..10: /note="n = A, C, G or U, or any modified base" /note="anticodon"
uuggacunnnaauucaa

SEQ ID NO: 26 - RNA, 18 nt, Artificial Sequence
  Anticodon arm
  misc_feature 8..11: /note="n = A, C, G or U, or any modified base" /note="extended (4nt) anticodon"
uuggacunnnnaauucaa

SEQ ID NO: 27 - RNA, 19 nt, Artificial Sequence
  Anticodon arm
  misc_feature 8..12: /note="n = A, C, G or U, or any modified base" /note="extended (5nt) anticodon"
uuggacunnnnnaauucaa

SEQ ID NO: 28 - RNA, 20 nt, Artificial Sequence
  Anticodon arm
  misc_feature 8..13: /note="n = A, C, G or U, or any modified base" /note="extended (6nt) anticodon"
uuggacunnnnnnaauucaa

SEQ ID NO: 29 - RNA, 17 nt, Artificial Sequence
  Anticodon arm
  misc_feature 8..10: /note="n = A, C, G or U, or any modified base" /note="anticodon"
auggucunnnaaaccau

SEQ ID NO: 30 - RNA, 18 nt, Artificial Sequence
  Anticodon arm
  misc_feature 8..11: /note="n = A, C, G or U, or any modified base" /note="extended (4nt) anticodon"
auggucunnnnaaaccau

SEQ ID NO: 31 - RNA, 19 nt, Artificial Sequence
  Anticodon arm
  misc_feature 8..12: /note="n = A, C, G or U, or any modified base" /note="extended (5nt) anticodon"
auggucunnnnnaaaccau

SEQ ID NO: 32 - RNA, 20 nt, Artificial Sequence
  Anticodon arm
  misc_feature 8..13: /note="n = A, C, G or U, or any modified base" /note="extended (6nt) anticodon"
auggucunnnnnnaaaccau

SEQ ID NO: 33 - RNA, 14 nt, Artificial Sequence
  v-loop
ugggguuuccccgc

SEQ ID NO: 34 - RNA, 14 nt, Artificial Sequence
  v-loop
aggggaaaccccgc

SEQ ID NO: 35 - RNA, 17 nt, Artificial Sequence
  T arm
  misc_feature 6..12: /note="T loop"
gcggguucgaaucccgu

SEQ ID NO: 36 - RNA, 17 nt, Artificial Sequence
  T arm
  misc_feature 6..12: /note="T loop"
acggguucgaaucccgu

SEQ ID NO: 37 - RNA, 17 nt, Artificial Sequence
  T arm
  misc_feature 6..12: /note="T loop"
gcggguucgagucccgu

SEQ ID NO: 38 - RNA, 17 nt, Artificial Sequence
  T arm
  misc_feature 6..12: /note="T loop"
acggguucgagucccgu